European Patent Specification EP 3 676 400 B1, published March 4, 2026. Title: EVALUATION OF PERFORMANCE OF COMPONENTS USING A PAIR OF DIMER-FORMING PRIMERS. Applicant: SEEGENE, INC. The sequence listing filed with the application follows.

SEQUENCE LISTING (12 sequences)

SEQ ID NO: 1 - DNA, 25 bp, Artificial Sequence
  Synthetic oligonucleotide: DFP-1
ttggcttggcttggctttagctgat

SEQ ID NO: 2 - DNA, 22 bp, Artificial Sequence
  Synthetic oligonucleotide: DFP-2
ggttctcaagcaacaatatcag

SEQ ID NO: 3 - DNA, 23 bp, Artificial Sequence
  Synthetic oligonucleotide: DFP-3
ggttctcaagcaacaatatcagc

SEQ ID NO: 4 - DNA, 24 bp, Artificial Sequence
  Synthetic oligonucleotide: DFP-4
ggttctcaagcaacaatatcagct

SEQ ID NO: 5 - DNA, 25 bp, Artificial Sequence
  Synthetic oligonucleotide: DFP-5
ttaccataccatacctttttgcgag

SEQ ID NO: 6 - DNA, 21 bp, Artificial Sequence
  Synthetic oligonucleotide: DFP-6
caatggatcggtatcactcgc

SEQ ID NO: 7 - DNA, 32 bp, Artificial Sequence
  Synthetic oligonucleotide: NG-F
tacgcctgctactttcacgctgtaatcagatg

SEQ ID NO: 8 - DNA, 32 bp, Artificial Sequence
  Synthetic oligonucleotide: NG-R
caatggatcggtatcactcgccgagcaagaac

SEQ ID NO: 9 - DNA, 22 bp, Artificial Sequence
  Synthetic oligonucleotide: NG-P
tgcccctcattggcgtgtttcg

SEQ ID NO: 10 - DNA, 36 bp, Artificial Sequence
  Synthetic oligonucleotide: CesA3-F
  misc_feature (22)..(26): n is deoxyinosine
atggaatccgaaggagaaaccnnnnnaaagccgatg

SEQ ID NO: 11 - DNA, 39 bp, Artificial Sequence
  Synthetic oligonucleotide: CesA3-R
  misc_feature (24)..(28): n is deoxyinosine
tcctctcatactcgtagcaaggcnnnnnaactgggaatg

SEQ ID NO: 12 - DNA, 23 bp, Artificial Sequence
  Synthetic oligonucleotide: CesA3-P
tctggcaagtctgcggaacaatg